European Patent Specification EP 3 725 883 B1, published January 24, 2024. Title: A method for production of an active form  GcMAF. Applicant: Nabeshima, Yoichi. The sequence listing filed with the application follows.

SEQUENCE LISTING (15 sequences)

SEQ ID NO: 1 - DNA, 1425 bp, Homo sapiens
atgaagagggtcctggtactactgcttgctgtggcatttggacatgctttagagagaggccgggattatgaaaagaataaagtctgcaaggaattctcccatctgggaaaggaggacttcacatctctgtcactagtcctgtacagtagaaaatttcccagtggcacgtttgaacaggtcagccaacttgtgaaggaagttgtctccttgaccgaagcctgctgtgcggaaggggctgaccctgactgctatgacaccaggacctcagcactgtctgccaagtcctgtgaaagtaattctccattccccgttcacccaggcactgctgagtgctgcaccaaagagggcctggaacgaaagctctgcatggctgctctgaaacaccagccacaggaattccctacctacgtggaacccacaaatgatgaaatctgtgaggcgttcaggaaagatccaaaggaatatgctaatcaatttatgtgggaatattccactaattacgaacaagctcctctgtcacttttagtcagttacaccaagagttatctttctatggtagggtcctgctgtacctctgcaagcccaactgtatgctttttgaaagagagactccagcttaaacatttatcacttctcaccactctgtcaaatagagtctgctcacaatatgctgcttatggggagaagaaatcaaggctcagcaatctcataaagttagcccaaaaagtgcctactgctgatctggaggatgttttgccactagctgaagatattactaacatcctctccaaatgctgtgagtctgcctctgaagattgcatggccaaagagctgcctgaacacacagtaaaactctgtgacaatttatccacaaagaattctaagtttgaagactgttgtcaagaaaaaacagccatggacgtttttgtgtgcacttacttcatgccagctgcccaactccccgagcttccagatgtaagattgcccacaaacaaagatgtgtgtgatccaggaaacaccaaagtcatggataagtatacatttgaactaagcagaaggactcatcttccggaagtattcctcagtaaggtacttgagccaaccctaaaaagccttggtgaatgctgtgatgttgaagactcaactacctgttttaatgctaagggccctctactaaagaaggaactatcttctttcattgacaagggacaagaactatgtgcagattattcagaaaatacatttactgagtacaagaaaaaactggcagagcgactaaaagcaaaattgcctgatgccacacccacggaactggcaaagctggttaacaagcactcagactttgcctccaactgctgttccataaactcacctcctctttactgtgattcagagattgatgctgaattgaagaatatcctgtag

SEQ ID NO: 2 - DNA, 1425 bp, Homo sapiens
atgaagagggtcctggtactactgcttgctgtggcatttggacatgctttagagagaggccgggattatgaaaagaataaagtctgcaaggaattctcccatctgggaaaggaggacttcacatctctgtcactagtcctgtacagtagaaaatttcccagtggcacgtttgaacaggtcagccaacttgtgaaggaagttgtctccttgaccgaagcctgctgtgcggaaggggctgaccctgactgctatgacaccaggacctcagcactgtctgccaagtcctgtgaaagtaattctccattccccgttcacccaggcactgctgagtgctgcaccaaagagggcctggaacgaaagctctgcatggctgctctgaaacaccagccacaggaattccctacctacgtggaacccacaaatgatgaaatctgtgaggcgttcaggaaagatccaaaggaatatgctaatcaatttatgtgggaatattccactaattacgaacaagctcctctgtcacttttagtcagttacaccaagagttatctttctatggtagggtcctgctgtacctctgcaagcccaactgtatgctttttgaaagagagactccagcttaaacatttatcacttctcaccactctgtcaaatagagtctgctcacaatatgctgcttatggggagaagaaatcaaggctcagcaatctcataaagttagcccaaaaagtgcctactgctgatctggaggatgttttgccactagctgaagatattactaacatcctctccaaatgctgtgagtctgcctctgaagattgcatggccaaagagctgcctgaacacacagtaaaactctgtgacaatttatccacaaagaattctaagtttgaagactgttgtcaagaaaaaacagccatggacgtttttgtgtgcacttacttcatgccagctgcccaactccccgagcttccagatgtaagattgcccacaaacaaagatgtgtgtgatccaggaaacaccaaagtcatggataagtatacatttgaactaagcagaaggactcatcttccggaagtattcctcagtaaggtacttgagccaaccctaaaaagccttggtgaatgctgtgatgttgaagactcaactacctgttttaatgctaagggccctctactaaagaaggaactatcttctttcattgacaagggacaagaactatgtgcagattattcagaaaatacatttactgagtacaagaaaaaactggcagagcgactaaaagcaaaattgcctgaggccacacccacggaactggcaaagctggttaacaagcactcagactttgcctccaactgctgttccataaactcacctcctctttactgtgattcagagattgatgctgaattgaagaatatcctgtag

SEQ ID NO: 3 - DNA, 1425 bp, Homo sapiens
atgaagagggtcctggtactactgcttgctgtggcatttggacatgctttagagagaggccgggattatgaaaagaataaagtctgcaaggaattctcccatctgggaaaggaggacttcacatctctgtcactagtcctgtacagtagaaaatttcccagtggcacgtttgaacaggtcagccaacttgtgaaggaagttgtctccttgaccgaagcctgctgtgcggaaggggctgaccctgactgctatgacaccaggacctcagcactgtctgccaagtcctgtgaaagtaattctccattccccgttcacccaggcactgctgagtgctgcaccaaagagggcctggaacgaaagctctgcatggctgctctgaaacaccagccacaggaattccctacctacgtggaacccacaaatgatgaaatctgtgaggcgttcaggaaagatccaaaggaatatgctaatcaatttatgtgggaatattccactaattacggacaagctcctctgtcacttttagtcagttacaccaagagttatctttctatggtagggtcctgctgtacctctgcaagcccaactgtatgctttttgaaagagagactccagcttaaacatttatcacttctcaccactctgtcaaatagagtctgctcacaatatgctgcttatggggagaagaaatcaaggctcagcaatctcataaagttagcccaaaaagtgcctactgctgatctggaggatgttttgccactagctgaagatattactaacatcctctccaaatgctgtgagtctgcctctgaagattgcatggccaaagagctgcctgaacacacagtaaaactctgtgacaatttatccacaaagaattctaagtttgaagactgttgtcaagaaaaaacagccatggacgtttttgtgtgcacttacttcatgccagctgcccaactccccgagcttccagatgtagagttgcccacaaacaaagatgtgtgtgatccaggaaacaccaaagtcatggataagtatacatttgaactaagcagaaggactcatcttccggaagtattcctcagtaaggtacttgagccaaccctaaaaagccttggtgaatgctgtgatgttgaagactcaactacctgttttaatgctaagggccctctactaaagaaggaactatcttctttcattgacaagggacaagaactatgtgcagattattcagaaaatacatttactgagtacaagaaaaaactggcagagcgactaaaagcaaaattgcctgatgccacacccaaggaactggcaaagctggttaacaagcactcagactttgcctccaactgctgttccataaactcacctcctctttactgtgattcagagattgatgctgaattgaagaatatcctgtag

SEQ ID NO: 4 - protein, 474 aa, Homo sapiens
MKRVLVLLLAVAFGHALERGRDYEKNKVCKEFSHLGKEDFTSLSLVLYSRKFPSGTFEQVSQLVKEVVSLTEACCAEGADPDCYDTRTSALSAKSCESNSPFPVHPGTAECCTKEGLERKLCMAALKHQPQEFPTYVEPTNDEICEAFRKDPKEYANQFMWEYSTNYEQAPLSLLVSYTKSYLSMVGSCCTSASPTVCFLKERLQLKHLSLLTTLSNRVCSQYAAYGEKKSRLSNLIKLAQKVPTADLEDVLPLAEDITNILSKCCESASEDCMAKELPEHTVKLCDNLSTKNSKFEDCCQEKTAMDVFVCTYFMPAAQLPELPDVRLPTNKDVCDPGNTKVMDKYTFELSRRTHLPEVFLSKVLEPTLKSLGECCDVEDSTTCFNAKGPLLKKELSSFIDKGQELCADYSENTFTEYKKKLAERLKAKLPDATPTELAKLVNKHSDFASNCCSINSPPLYCDSEIDAELKNIL

SEQ ID NO: 5 - protein, 474 aa, Homo sapiens
MKRVLVLLLAVAFGHALERGRDYEKNKVCKEFSHLGKEDFTSLSLVLYSRKFPSGTFEQVSQLVKEVVSLTEACCAEGADPDCYDTRTSALSAKSCESNSPFPVHPGTAECCTKEGLERKLCMAALKHQPQEFPTYVEPTNDEICEAFRKDPKEYANQFMWEYSTNYEQAPLSLLVSYTKSYLSMVGSCCTSASPTVCFLKERLQLKHLSLLTTLSNRVCSQYAAYGEKKSRLSNLIKLAQKVPTADLEDVLPLAEDITNILSKCCESASEDCMAKELPEHTVKLCDNLSTKNSKFEDCCQEKTAMDVFVCTYFMPAAQLPELPDVRLPTNKDVCDPGNTKVMDKYTFELSRRTHLPEVFLSKVLEPTLKSLGECCDVEDSTTCFNAKGPLLKKELSSFIDKGQELCADYSENTFTEYKKKLAERLKAKLPEATPTELAKLVNKHSDFASNCCSINSPPLYCDSEIDAELKNIL

SEQ ID NO: 6 - protein, 474 aa, Homo sapiens
MKRVLVLLLAVAFGHALERGRDYEKNKVCKEFSHLGKEDFTSLSLVLYSRKFPSGTFEQVSQLVKEVVSLTEACCAEGADPDCYDTRTSALSAKSCESNSPFPVHPGTAECCTKEGLERKLCMAALKHQPQEFPTYVEPTNDEICEAFRKDPKEYANQFMWEYSTNYGQAPLSLLVSYTKSYLSMVGSCCTSASPTVCFLKERLQLKHLSLLTTLSNRVCSQYAAYGEKKSRLSNLIKLAQKVPTADLEDVLPLAEDITNILSKCCESASEDCMAKELPEHTVKLCDNLSTKNSKFEDCCQEKTAMDVFVCTYFMPAAQLPELPDVELPTNKDVCDPGNTKVMDKYTFELSRRTHLPEVFLSKVLEPTLKSLGECCDVEDSTTCFNAKGPLLKKELSSFIDKGQELCADYSENTFTEYKKKLAERLKAKLPDATPKELAKLVNKHSDFASNCCSINSPPLYCDSEIDAELKNIL

SEQ ID NO: 7 - DNA, 1425 bp, Homo sapiens
atgaagcgggtgctggtgctgctgctggccgtggcctttggacacgccctggaaagaggccgggactacgagaagaacaaagtgtgcaaagagttcagccacctgggcaaagaggacttcaccagcctgagcctggtgctgtacagccggaagttccccagcggcaccttcgaacaggtgtcccagctggtcaaagaagtggtgtccctgaccgaggcctgttgcgccgaaggcgccgaccctgactgctacgataccagaacaagcgccctgagcgccaagagctgcgagagcaacagcccctttcctgtgcaccctggcaccgccgagtgctgcacaaaagagggcctggaacggaagctgtgcatggccgccctgaagcaccagccccaggaattccctacctacgtcgagcccaccaacgacgagatttgcgaggccttcagaaaggaccccaaagagtacgccaaccagttcatgtgggagtacagcaccaactacgagcaggcccccctgagcctgctggtgtcctacaccaagagctacctgagcatggtcggaagctgctgcaccagcgccagccctaccgtgtgcttcctgaaagagcggctgcagctgaagcacctgtccctgctgaccaccctgagcaacagagtgtgcagccagtacgccgcctacggcgagaagaagtcccggctgagcaacctgatcaagctggcccagaaggtgcccaccgccgacctggaagatgtgctgcctctggccgaggacatcaccaacatcctgagcaagtgctgcgagtccgccagcgaggactgcatggccaaagagctgcccgagcacaccgtgaagctgtgcgacaacctgagcaccaagaacagcaagttcgaggactgctgccaggaaaagaccgccatggacgtgttcgtgtgcacctacttcatgcctgccgcccagctgcctgagctgccagatgtgcggctgcccaccaacaaggacgtgtgcgaccccggcaacaccaaagtgatggacaagtacaccttcgagctgagccggcggacccatctgcccgaagtgtttctgtccaaggtgctggaacccaccctgaagtccctgggcgagtgctgcgacgtggaagatagcaccacctgtttcaacgccaagggccccctgctgaagaaagagctgagcagcttcatcgacaagggccaggaactgtgcgccgactacagcgagaacaccttcaccgagtacaagaagaagctggccgagcggctgaaggccaagctgcctgatgccacacctaccgagctggccaagctggtcaacaagcggagcgacttcgccagcaactgctgcagcatcaacagccccccactgtactgcgacagcgagatcgacgccgagctgaagaacatcctgtag

SEQ ID NO: 8 - protein, 474 aa, Homo sapiens
MKRVLVLLLAVAFGHALERGRDYEKNKVCKEFSHLGKEDFTSLSLVLYSRKFPSGTFEQVSQLVKEVVSLTEACCAEGADPDCYDTRTSALSAKSCESNSPFPVHPGTAECCTKEGLERKLCMAALKHQPQEFPTYVEPTNDEICEAFRKDPKEYANQFMWEYSTNYEQAPLSLLVSYTKSYLSMVGSCCTSASPTVCFLKERLQLKHLSLLTTLSNRVCSQYAAYGEKKSRLSNLIKLAQKVPTADLEDVLPLAEDITNILSKCCESASEDCMAKELPEHTVKLCDNLSTKNSKFEDCCQEKTAMDVFVCTYFMPAAQLPELPDVRLPTNKDVCDPGNTKVMDKYTFELSRRTHLPEVFLSKVLEPTLKSLGECCDVEDSTTCFNAKGPLLKKELSSFIDKGQELCADYSENTFTEYKKKLAERLKAKLPDATPTELAKLVNKRSDFASNCCSINSPPLYCDSEIDAELKNIL

SEQ ID NO: 9 - DNA, 1458 bp, Homo sapiens
atgaagcgggtgctggtgctgctgctggccgtggcctttggacacgccctggaaagaggccgggactacgagaagaacaaagtgtgcaaagagttcagccacctgggcaaagaggacttcaccagcctgagcctggtgctgtacagccggaagttccccagcggcaccttcgaacaggtgtcccagctggtcaaagaagtggtgtccctgaccgaggcctgttgcgccgaaggcgccgaccctgactgctacgataccagaacaagcgccctgagcgccaagagctgcgagagcaacagcccctttcctgtgcaccctggcaccgccgagtgctgcacaaaagagggcctggaacggaagctgtgcatggccgccctgaagcaccagccccaggaattccctacctacgtcgagcccaccaacgacgagatttgcgaggccttcagaaaggaccccaaagagtacgccaaccagttcatgtgggagtacagcaccaactacgagcaggcccccctgagcctgctggtgtcctacaccaagagctacctgagcatggtcggaagctgctgcaccagcgccagccctaccgtgtgcttcctgaaagagcggctgcagctgaagcacctgtccctgctgaccaccctgagcaacagagtgtgcagccagtacgccgcctacggcgagaagaagtcccggctgagcaacctgatcaagctggcccagaaggtgcccaccgccgacctggaagatgtgctgcctctggccgaggacatcaccaacatcctgagcaagtgctgcgagtccgccagcgaggactgcatggccaaagagctgcccgagcacaccgtgaagctgtgcgacaacctgagcaccaagaacagcaagttcgaggactgctgccaggaaaagaccgccatggacgtgttcgtgtgcacctacttcatgcctgccgcccagctgcctgagctgccagatgtgcggctgcccaccaacaaggacgtgtgcgaccccggcaacaccaaagtgatggacaagtacaccttcgagctgagccggcggacccatctgcccgaagtgtttctgtccaaggtgctggaacccaccctgaagtccctgggcgagtgctgcgacgtggaagatagcaccacctgtttcaacgccaagggccccctgctgaagaaagagctgagcagcttcatcgacaagggccaggaactgtgcgccgactacagcgagaacaccttcaccgagtacaagaagaagctggccgagcggctgaaggccaagctgcctgatgccacacctaccgagctggccaagctggtcaacaagcggagcgacttcgccagcaactgctgcagcatcaacagccccccactgtactgcgacagcgagatcgacgccgagctgaagaacatcctgcaccaccaccatcaccatcatcaccaccattgatga

SEQ ID NO: 10 - DNA, 1428 bp, Homo sapiens
atgaagcgggtgctggtgctgctgctggccgtggcctttggacacgccctggaaagaggccgggactacgagaagaacaaagtgtgcaaagagttcagccacctgggcaaagaggacttcaccagcctgagcctggtgctgtacagccggaagttccccagcggcaccttcgaacaggtgtcccagctggtcaaagaagtggtgtccctgaccgaggcctgttgcgccgaaggcgccgaccctgactgctacgataccagaacaagcgccctgagcgccaagagctgcgagagcaacagcccctttcctgtgcaccctggcaccgccgagtgctgcacaaaagagggcctggaacggaagctgtgcatggccgccctgaagcaccagccccaggaattccctacctacgtcgagcccaccaacgacgagatttgcgaggccttcagaaaggaccccaaagagtacgccaaccagttcatgtgggagtacagcaccaactacgagcaggcccccctgagcctgctggtgtcctacaccaagagctacctgagcatggtcggaagctgctgcaccagcgccagccctaccgtgtgcttcctgaaagagcggctgcagctgaagcacctgtccctgctgaccaccctgagcaacagagtgtgcagccagtacgccgcctacggcgagaagaagtcccggctgagcaacctgatcaagctggcccagaaggtgcccaccgccgacctggaagatgtgctgcctctggccgaggacatcaccaacatcctgagcaagtgctgcgagtccgccagcgaggactgcatggccaaagagctgcccgagcacaccgtgaagctgtgcgacaacctgagcaccaagaacagcaagttcgaggactgctgccaggaaaagaccgccatggacgtgttcgtgtgcacctacttcatgcctgccgcccagctgcctgagctgccagatgtgcggctgcccaccaacaaggacgtgtgcgaccccggcaacaccaaagtgatggacaagtacaccttcgagctgagccggcggacccatctgcccgaagtgtttctgtccaaggtgctggaacccaccctgaagtccctgggcgagtgctgcgacgtggaagatagcaccacctgtttcaacgccaagggccccctgctgaagaaagagctgagcagcttcatcgacaagggccaggaactgtgcgccgactacagcgagaacaccttcaccgagtacaagaagaagctggccgagcggctgaaggccaagctgcctgaggccacacctaccgagctggccaagctggtcaacaagcggagcgacttcgccagcaactgctgcagcatcaacagccccccactgtactgcgacagcgagatcgacgccgagctgaagaacatcctgtgatga

SEQ ID NO: 11 - protein, 474 aa, Homo sapiens [sequence omitted]

SEQ ID NO: 12 - DNA, 1428 bp, Homo sapiens
atgaagcgggtgctggtgctgctgctggccgtggcctttggacacgccctggaaagaggccgggactacgagaagaacaaagtgtgcaaagagttcagccacctgggcaaagaggacttcaccagcctgagcctggtgctgtacagccggaagttccccagcggcaccttcgaacaggtgtcccagctggtcaaagaagtggtgtccctgaccgaggcctgttgcgccgaaggcgccgaccctgactgctacgataccagaacaagcgccctgagcgccaagagctgcgagagcaacagcccctttcctgtgcaccctggcaccgccgagtgctgcacaaaagagggcctggaacggaagctgtgcatggccgccctgaagcaccagccccaggaattccctacctacgtcgagcccaccaacgacgagatttgcgaggccttcagaaaggaccccaaagagtacgccaaccagttcatgtgggagtacagcaccaactacgagcaggcccccctgagcctgctggtgtcctacaccaagagctacctgagcatggtcggaagctgctgcaccagcgccagccctaccgtgtgcttcctgaaagagcggctgcagctgaagcacctgtccctgctgaccaccctgagcaacagagtgtgcagccagtacgccgcctacggcgagaagaagtcccggctgagcaacctgatcaagctggcccagaaggtgcccaccgccgacctggaagatgtgctgcctctggccgaggacatcaccaacatcctgagcaagtgctgcgagtccgccagcgaggactgcatggccaaagagctgcccgagcacaccgtgaagctgtgcgacaacctgagcaccaagaacagcaagttcgaggactgctgccaggaaaagaccgccatggacgtgttcgtgtgcacctacttcatgcctgccgcccagctgcctgagctgccagatgtgcggctgcccaccaacaaggacgtgtgcgaccccggcaacaccaaagtgatggacaagtacaccttcgagctgagccggcggacccatctgcccgaagtgtttctgtccaaggtgctggaacccaccctgaagtccctgggcgagtgctgcgacgtggaagatagcaccacctgtttcaacgccaagggccccctgctgaagaaagagctgagcagcttcatcgacaagggccaggaactgtgcgccgactacagcgagaacaccttcaccgagtacaagaagaagctggccgagcggctgaaggccaagctgcctgatgccacacctaaggagctggccaagctggtcaacaagcggagcgacttcgccagcaactgctgcagcatcaacagccccccactgtactgcgacagcgagatcgacgccgagctgaagaacatcctgtgatga

SEQ ID NO: 13 - protein, 474 aa, Homo sapiens
MKRVLVLLLAVAFGHALERGRDYEKNKVCKEFSHLGKEDFTSLSLVLYSRKFPSGTFEQVSQLVKEVVSLTEACCAEGADPDCYDTRTSALSAKSCESNSPFPVHPGTAECCTKEGLERKLCMAALKHQPQEFPTYVEPTNDEICEAFRKDPKEYANQFMWEYSTNYEQAPLSLLVSYTKSYLSMVGSCCTSASPTVCFLKERLQLKHLSLLTTLSNRVCSQYAAYGEKKSRLSNLIKLAQKVPTADLEDVLPLAEDITNILSKCCESASEDCMAKELPEHTVKLCDNLSTKNSKFEDCCQEKTAMDVFVCTYFMPAAQLPELPDVRLPTNKDVCDPGNTKVMDKYTFELSRRTHLPEVFLSKVLEPTLKSLGECCDVEDSTTCFNAKGPLLKKELSSFIDKGQELCADYSENTFTEYKKKLAERLKAKLPDATPKELAKLVNKRSDFASNCCSINSPPLYCDSEIDAELKNIL

SEQ ID NO: 14 - DNA, 1458 bp, Homo sapiens
atgaagcgggtgctggtgctgctgctggccgtggcctttggacacgccctggaaagaggccgggactacgagaagaacaaagtgtgcaaagagttcagccacctgggcaaagaggacttcaccagcctgagcctggtgctgtacagccggaagttccccagcggcaccttcgaacaggtgtcccagctggtcaaagaagtggtgtccctgaccgaggcctgttgcgccgaaggcgccgaccctgactgctacgataccagaacaagcgccctgagcgccaagagctgcgagagcaacagcccctttcctgtgcaccctggcaccgccgagtgctgcacaaaagagggcctggaacggaagctgtgcatggccgccctgaagcaccagccccaggaattccctacctacgtcgagcccaccaacgacgagatttgcgaggccttcagaaaggaccccaaagagtacgccaaccagttcatgtgggagtacagcaccaactacgagcaggcccccctgagcctgctggtgtcctacaccaagagctacctgagcatggtcggaagctgctgcaccagcgccagccctaccgtgtgcttcctgaaagagcggctgcagctgaagcacctgtccctgctgaccaccctgagcaacagagtgtgcagccagtacgccgcctacggcgagaagaagtcccggctgagcaacctgatcaagctggcccagaaggtgcccaccgccgacctggaagatgtgctgcctctggccgaggacatcaccaacatcctgagcaagtgctgcgagtccgccagcgaggactgcatggccaaagagctgcccgagcacaccgtgaagctgtgcgacaacctgagcaccaagaacagcaagttcgaggactgctgccaggaaaagaccgccatggacgtgttcgtgtgcacctacttcatgcctgccgcccagctgcctgagctgccagatgtgcggctgcccaccaacaaggacgtgtgcgaccccggcaacaccaaagtgatggacaagtacaccttcgagctgagccggcggacccatctgcccgaagtgtttctgtccaaggtgctggaacccaccctgaagtccctgggcgagtgctgcgacgtggaagatagcaccacctgtttcaacgccaagggccccctgctgaagaaagagctgagcagcttcatcgacaagggccaggaactgtgcgccgactacagcgagaacaccttcaccgagtacaagaagaagctggccgagcggctgaaggccaagctgcctgaggccacacctaccgagctggccaagctggtcaacaagcggagcgacttcgccagcaactgctgcagcatcaacagccccccactgtactgcgacagcgagatcgacgccgagctgaagaacatcctgcaccaccaccatcaccatcatcaccaccattgatga

SEQ ID NO: 15 - DNA, 1458 bp, Homo sapiens
atgaagcgggtgctggtgctgctgctggccgtggcctttggacacgccctggaaagaggccgggactacgagaagaacaaagtgtgcaaagagttcagccacctgggcaaagaggacttcaccagcctgagcctggtgctgtacagccggaagttccccagcggcaccttcgaacaggtgtcccagctggtcaaagaagtggtgtccctgaccgaggcctgttgcgccgaaggcgccgaccctgactgctacgataccagaacaagcgccctgagcgccaagagctgcgagagcaacagcccctttcctgtgcaccctggcaccgccgagtgctgcacaaaagagggcctggaacggaagctgtgcatggccgccctgaagcaccagccccaggaattccctacctacgtcgagcccaccaacgacgagatttgcgaggccttcagaaaggaccccaaagagtacgccaaccagttcatgtgggagtacagcaccaactacgagcaggcccccctgagcctgctggtgtcctacaccaagagctacctgagcatggtcggaagctgctgcaccagcgccagccctaccgtgtgcttcctgaaagagcggctgcagctgaagcacctgtccctgctgaccaccctgagcaacagagtgtgcagccagtacgccgcctacggcgagaagaagtcccggctgagcaacctgatcaagctggcccagaaggtgcccaccgccgacctggaagatgtgctgcctctggccgaggacatcaccaacatcctgagcaagtgctgcgagtccgccagcgaggactgcatggccaaagagctgcccgagcacaccgtgaagctgtgcgacaacctgagcaccaagaacagcaagttcgaggactgctgccaggaaaagaccgccatggacgtgttcgtgtgcacctacttcatgcctgccgcccagctgcctgagctgccagatgtgcggctgcccaccaacaaggacgtgtgcgaccccggcaacaccaaagtgatggacaagtacaccttcgagctgagccggcggacccatctgcccgaagtgtttctgtccaaggtgctggaacccaccctgaagtccctgggcgagtgctgcgacgtggaagatagcaccacctgtttcaacgccaagggccccctgctgaagaaagagctgagcagcttcatcgacaagggccaggaactgtgcgccgactacagcgagaacaccttcaccgagtacaagaagaagctggccgagcggctgaaggccaagctgcctgatgccacacctaaggagctggccaagctggtcaacaagcggagcgacttcgccagcaactgctgcagcatcaacagccccccactgtactgcgacagcgagatcgacgccgagctgaagaacatcctgcaccaccaccatcaccatcatcaccaccattgatga